European Patent Application EP 4 350 003 A1, published April 10, 2024. Title: Low input chromosome conformation capture methods. Applicant: FUNDACIÓ INSTITUT DE RECERCA CONTRA LA LEUCÈMIA JOSEP CARRERAS. The sequence listing filed with the application follows.

SEQUENCE LISTING (4 sequences)

SEQ ID NO: 1 - DNA, 32 bp, synthetic construct
  source 1..32: mol_type = other DNA
gatcggaagagcggttcagcaggaatgccgag

SEQ ID NO: 2 - DNA, 33 bp, synthetic construct
  source 1..33: mol_type = other DNA
acactctttccctacacgacgctcttccgatct

SEQ ID NO: 3 - DNA, 58 bp, synthetic construct
  source 1..58: mol_type = other DNA
aatgatacggcgaccaccgagatctacactctttccctacacgacgctcttccgatct

SEQ ID NO: 4 - DNA, 61 bp, synthetic construct
  source 1..61: mol_type = other DNA
caagcagaagacggcatacgagatcggtctcggcattcctgctgaaccgctcttccgatct